European Patent Specification EP 3 828 263 B1, published February 15, 2023. Title: Method and kit for preparing clinical-grade mesenchymal stem cells derived from human induced pluripotent stem cells. Applicant: Shanghai Oriental Hospital(affiliated East Hospital of Tongji University). The sequence listing filed with the application follows.

SEQUENCE LISTING (10 sequences)

SEQ ID NO: 1 - DNA, 19 bp, Artificial Sequence
  hTGFβ_Forward
ggccagatcctgtccaagc

SEQ ID NO: 2 - DNA, 21 bp, Artificial Sequence
  hTGFβ_Revers
gtgggtttccaccattagcac

SEQ ID NO: 3 - DNA, 21 bp, Artificial Sequence
  hIL-6_ Forward
cctgaaccttccaaagatggc

SEQ ID NO: 4 - DNA, 21 bp, Artificial Sequence
  hIL-6_ Revers
ttcaccaggcaagtctcctca

SEQ ID NO: 5 - DNA, 21 bp, Artificial Sequence
  hIDO1_ Forward
gccagcttcgagaaagagttg

SEQ ID NO: 6 - DNA, 21 bp, Artificial Sequence
  hIDO1_ Revers
atcccagaactagacgtgcaa

SEQ ID NO: 7 - DNA, 19 bp, Artificial Sequence
  hPGE2_ Forward
cgatgctcatgctcttcgc

SEQ ID NO: 8 - DNA, 22 bp, Artificial Sequence
  hPGE2_ Revers
gggagactgcatagatgacagg

SEQ ID NO: 9 - DNA, 23 bp, Artificial Sequence
  hIL-10_ Forward
gactttaagggttacctgggttg

SEQ ID NO: 10 - DNA, 21 bp, Artificial Sequence
  hIL-10_ Revers
tcacatgcgccttgatgtctg